European Patent Application EP 4 112 642 A1, published January 4, 2023. Title: ANTI-CD137 CONSTRUCTS AND USES THEREOF. Applicant: SHANGHAI HENLIUS BIOTECH, INC. The sequence listing filed with the application follows.

SEQUENCE LISTING (230 sequences)

SEQ ID NO: 1 - protein, 5 aa, Artificial Sequence
  DOMAIN (1)..(5): Clone 3 VH CDR1
DTYIH

SEQ ID NO: 2 - protein, 17 aa, Artificial Sequence
  DOMAIN (1)..(17): Clone 3 VH CDR2
RIDPANGFTEYAQKFQG

SEQ ID NO: 3 - protein, 10 aa, Artificial Sequence
  DOMAIN (1)..(10): Clone 3 VH CDR3
GNLHYALMDY

SEQ ID NO: 4 - protein, 11 aa, Artificial Sequence
  DOMAIN (1)..(11): Clone 3 VL CDR1
KASQAINTYLS

SEQ ID NO: 5 - protein, 7 aa, Artificial Sequence
  DOMAIN (1)..(7): Clone 3 VL CDR2
RANRMVD

SEQ ID NO: 6 - protein, 9 aa, Artificial Sequence
  DOMAIN (1)..(9): Clone 3 VL CDR3
LQSDDFPYT

SEQ ID NO: 7 - protein, 119 aa, Artificial Sequence
  DOMAIN (1)..(119): Clone 3 VH
QVQLVQSGAEVKKPGASVKVSCKASGFNPKDTYIHWVRQAPGQGLEWMGRIDPANGFTEYAQKFQGRVTMTRDTSTSTVYMELSSLRSEDTAVYYCTTGNLHYALMDYWGQGTSVTVSS

SEQ ID NO: 8 - protein, 110 aa, Artificial Sequence
  DOMAIN (1)..(110): Clone 3 VL
DIQMTQSPSSVSASVGDRVTITCKASQAINTYLSWYQQKPGKAPKLLIYRANRMVDGVPSRFSGSGSGTDFTLTISSLQHEDFATYYCLQSDDFPYTFGGGTKLEIKRTV

SEQ ID NO: 9 - protein, 445 aa, Artificial Sequence
  CHAIN (1)..(445): Clone 3 HC
QVQLVQSGAEVKKPGASVKVSCKASGFNPKDTYIHWVRQAPGQGLEWMGRIDPANGFTEYAQKFQGRVTMTRDTSTSTVYMELSSLRSEDTAVYYCTTGNLHYALMDYWGQGTSVTVSSASTKGPSVFPLAPCSRSTSESTAALGCLVKDYFPEPVTVSWNSGALTSGVHTFPAVLQSSGLYSLSSVVTVPSSNFGTQTYTCNVDHKPSNTKVDKTVERKCCVECPPCPAPPVAGPSVFLFPPKPKDTLMISRTPEVTCVVVDVSHEDPEVQFNWYVDGVEVHNAKTKPREEQFNSTFRVVSVLTVVHQDWLNGKEYKCKVSNKGLPAPIEKTISKTKGQPREPQVYTLPPSREEMTKNQVSLTCLVKGFYPSDIAVEWESNGQPENNYKTTPPMLDSDGSFFLYSKLTVDKSRWQQGNVFSCSVMHEALHNHYTQKSLSLSPGK

SEQ ID NO: 10 - protein, 214 aa, Artificial Sequence
  CHAIN (1)..(214): Clone 3 LC
DIQMTQSPSSVSASVGDRVTITCKASQAINTYLSWYQQKPGKAPKLLIYRANRMVDGVPSRFSGSGSGTDFTLTISSLQHEDFATYYCLQSDDFPYTFGGGTKLEIKRTVAAPSVFIFPPSDEQLKSGTASVVCLLNNFYPREAKVQWKVDNALQSGNSQESVTEQDSKDSTYSLSSTLTLSKADYEKHKVYACEVTHQGLSSPVTKSFNRGEC

SEQ ID NO: 11 - protein, 5 aa, Artificial Sequence
  DOMAIN (1)..(5): Clone 9 VH CDR1
DTYIH

SEQ ID NO: 12 - protein, 17 aa, Artificial Sequence
  DOMAIN (1)..(17): Clone 9 VH CDR2
KIDPANGNTEYAQKFQG

SEQ ID NO: 13 - protein, 10 aa, Artificial Sequence
  DOMAIN (1)..(10): Clone 9 VH CDR3
GNLHYALMDY

SEQ ID NO: 14 - protein, 11 aa, Artificial Sequence
  DOMAIN (1)..(11): Clone 9 VL CDR1
KASQAIATYLS

SEQ ID NO: 15 - protein, 7 aa, Artificial Sequence
  DOMAIN (1)..(7): Clone 9 VL CDR2
RANRMYD

SEQ ID NO: 16 - protein, 9 aa, Artificial Sequence
  DOMAIN (1)..(9): Clone 9 VL CDR3
LQFDDFPYT

SEQ ID NO: 17 - protein, 119 aa, Artificial Sequence
  DOMAIN (1)..(119): Clone 9 VH
QVQLVQSGAEVKKPGASVKVSCKASGFNLKDTYIHWVRQAPGQGLEWMGKIDPANGNTEYAQKFQGRVTMTRDTSTSTVYMELSSLRSEDTAVYYCTTGNLHYALMDYWGQGTSVTVSS

SEQ ID NO: 18 - protein, 110 aa, Artificial Sequence
  DOMAIN (1)..(110): Clone 9 VL
DIQMTQSPSSVSASVGDRVTITCKASQAIATYLSWYQQKPGKAPKLLIYRANRMYDGVPSRFSGSGSGTDFTLTISSLQPEDFATYYCLQFDDFPYTFGGGTKLEIKRTV

SEQ ID NO: 19 - protein, 445 aa, Artificial Sequence
  CHAIN (1)..(445): Clone 9 HC
QVQLVQSGAEVKKPGASVKVSCKASGFNLKDTYIHWVRQAPGQGLEWMGKIDPANGNTEYAQKFQGRVTMTRDTSTSTVYMELSSLRSEDTAVYYCTTGNLHYALMDYWGQGTSVTVSSASTKGPSVFPLAPCSRSTSESTAALGCLVKDYFPEPVTVSWNSGALTSGVHTFPAVLQSSGLYSLSSVVTVPSSNFGTQTYTCNVDHKPSNTKVDKTVERKCCVECPPCPAPPVAGPSVFLFPPKPKDTLMISRTPEVTCVVVDVSHEDPEVQFNWYVDGVEVHNAKTKPREEQFNSTFRVVSVLTVVHQDWLNGKEYKCKVSNKGLPAPIEKTISKTKGQPREPQVYTLPPSREEMTKNQVSLTCLVKGFYPSDIAVEWESNGQPENNYKTTPPMLDSDGSFFLYSKLTVDKSRWQQGNVFSCSVMHEALHNHYTQKSLSLSPGK

SEQ ID NO: 20 - protein, 214 aa, Artificial Sequence
  CHAIN (1)..(214): Clone 9 LC
DIQMTQSPSSVSASVGDRVTITCKASQAIATYLSWYQQKPGKAPKLLIYRANRMYDGVPSRFSGSGSGTDFTLTISSLQPEDFATYYCLQFDDFPYTFGGGTKLEIKRTVAAPSVFIFPPSDEQLKSGTASVVCLLNNFYPREAKVQWKVDNALQSGNSQESVTEQDSKDSTYSLSSTLTLSKADYEKHKVYACEVTHQGLSSPVTESLNRGEC

SEQ ID NO: 21 - protein, 5 aa, Artificial Sequence
  DOMAIN (1)..(5): Clone 23 VH CDR1
DTYIH

SEQ ID NO: 22 - protein, 17 aa, Artificial Sequence
  DOMAIN (1)..(17): Clone 23 VH CDR2
KIDPANGQTEYAQKFQG

SEQ ID NO: 23 - protein, 10 aa, Artificial Sequence
  DOMAIN (1)..(10): Clone 23 VH CDR3
GNLHYALMDY

SEQ ID NO: 24 - protein, 11 aa, Artificial Sequence
  DOMAIN (1)..(11): Clone 23 VL CDR1
KASQAINTYLS

SEQ ID NO: 25 - protein, 7 aa, Artificial Sequence
  DOMAIN (1)..(7): Clone 23 VL CDR2
RANRMVG

SEQ ID NO: 26 - protein, 9 aa, Artificial Sequence
  DOMAIN (1)..(9): Clone 23 VL CDR3
LQYRDFPYT

SEQ ID NO: 27 - protein, 119 aa, Artificial Sequence
  DOMAIN (1)..(119): Clone 23 VH
QVQLVQSGAEVKKPGASVKVSCKASGFNIKDTYIHWVRQAPGQGLEWMGKIDPANGQTEYAQKFQGRVTMTRDTSTSTVYMELSSLRSEDTAVYYCTTGNLHYALMDYWGQGTSVTVSS

SEQ ID NO: 28 - protein, 110 aa, Artificial Sequence
  DOMAIN (1)..(110): Clone 23 VL
DIQMTQSPSSVSASVGDRVTITCKASQAINTYLSWYQQKPGKAPKLLIYRANRMVGGVPSRFSGSGSGTDFTLTISSLQPEDFATYYCLQYRDFPYTFGGGTKLEIKRTV

SEQ ID NO: 29 - protein, 445 aa, Artificial Sequence
  CHAIN (1)..(445): Clone 23 HC
QVQLVQSGAEVKKPGASVKVSCKASGFNIKDTYIHWVRQAPGQGLEWMGKIDPANGQTEYAQKFQGRVTMTRDTSTSTVYMELSSLRSEDTAVYYCTTGNLHYALMDYWGQGTSVTVSSASTKGPSVFPLAPCSRSTSESTAALGCLVKDYFPEPVTVSWNSGALTSGVHTFPAVLQSSGLYSLSSVVTVPSSNFGTQTYTCNVDHKPSNTKVDKTVERKCCVECPPCPAPPVAGPSVFLFPPKPKDTLMISRTPEVTCVVVDVSHEDPEVQFNWYVDGVEVHNAKTKPREEQFNSTFRVVSVLTVVHQDWLNGKEYKCKVSNKGLPAPIEKTISKTKGQPREPQVYTLPPSREEMTKNQVSLTCLVKGFYPSDIAVEWESNGQPENNYKTTPPMLDSDGSFFLYSKLTVDKSRWQQGNVFSCSVMHEALHNHYTQKSLSLSPGK

SEQ ID NO: 30 - protein, 214 aa, Artificial Sequence
  CHAIN (1)..(214): Clone 23 LC
DIQMTQSPSSVSASVGDRVTITCKASQAINTYLSWYQQKPGKAPKLLIYRANRMVGGVPSRFSGSGSGTDFTLTISSLQPEDFATYYCLQYRDFPYTFGGGTKLEIKRTVAAPSVFIFPPSDEQLKSGTASVVCLLNNFYPREAKVQWKVDNALQSGNSQESVTEQDSKDSTYSLSSTLTLSKADYEKHKVYACEVTHQGLSSPVTKSFNRGEC

SEQ ID NO: 31 - protein, 5 aa, Artificial Sequence
  DOMAIN (1)..(5): Clone 25 VH CDR1
DTYIH

SEQ ID NO: 32 - protein, 17 aa, Artificial Sequence
  DOMAIN (1)..(17): Clone 25 VH CDR2
RIDPANGNSEYAQKFQG

SEQ ID NO: 33 - protein, 10 aa, Artificial Sequence
  DOMAIN (1)..(10): Clone 25 VH CDR3
GNLHYGLMDY

SEQ ID NO: 34 - protein, 11 aa, Artificial Sequence
  DOMAIN (1)..(11): Clone 25 VL CDR1
KASQAINTYLS

SEQ ID NO: 35 - protein, 7 aa, Artificial Sequence
  DOMAIN (1)..(7): Clone 25 VL CDR2
RDNRKVD

SEQ ID NO: 36 - protein, 9 aa, Artificial Sequence
  DOMAIN (1)..(9): Clone 25 VL CDR3
LQYQDFPYK

SEQ ID NO: 37 - protein, 119 aa, Artificial Sequence
  DOMAIN (1)..(119): Clone 25 VH
QVQLVQSGAEVKKPGASVKVSCKASGFNIQDTYIHWVRQAPGQGLEWMGRIDPANGNSEYAQKFQGRVTMTRDTSTSTVYMELSSLRSEDTAVYYCTTGNLHYGLMDYWGQGTSVTVSS

SEQ ID NO: 38 - protein, 110 aa, Artificial Sequence
  DOMAIN (1)..(110): Clone 25 VL
DIQMTQSPSSVSASVGDRVTITCKASQAINTYLSWYQQKPGKAPKLLIYRDNRKVDGVPSRFSGSGSGTDFTLTISSLQPEDFATYYCLQYQDFPYKFGGGTKLEIKRTV

SEQ ID NO: 39 - protein, 445 aa, Artificial Sequence
  CHAIN (1)..(445): Clone 25 HC
QVQLVQSGAEVKKPGASVKVSCKASGFNIQDTYIHWVRQAPGQGLEWMGRIDPANGNSEYAQKFQGRVTMTRDTSTSTVYMELSSLRSEDTAVYYCTTGNLHYGLMDYWGQGTSVTVSSASTKGPSVFPLAPCSRSTSESTAALGCLVKDYFPEPVTVSWNSGALTSGVHTFPAVLQSSGLYSLSSVVTVPSSNFGTQTYTCNVDHKPSNTKVDKTVERKCCVECPPCPAPPVAGPSVFLFPPKPKDTLMISRTPEVTCVVVDVSHEDPEVQFNWYVDGVEVHNAKTKPREEQFNSTFRVVSVLTVVHQDWLNGKEYKCKVSNKGLPAPIEKTISKTKGQPREPQVYTLPPSREEMTKNQVSLTCLVKGFYPSDIAVEWESNGQPENNYKTTPPMLDSDGSFFLYSKLTVDKSRWQQGNVFSCSVMHEALHNHYTQKSLSLSPGK

SEQ ID NO: 40 - protein, 214 aa, Artificial Sequence
  CHAIN (1)..(214): Clone 25 LC
DIQMTQSPSSVSASVGDRVTITCKASQAINTYLSWYQQKPGKAPKLLIYRDNRKVDGVPSRFSGSGSGTDFTLTISSLQPEDFATYYCLQYQDFPYKFGGGTKLEIKRTVAAPSVFIFPPSDEQLKSGTASVVCLLNNFYPREAKVQWKVDNALQSGNSQESVTEQDSKDSTYSLSSTLTLSKADYEKHKVYACEVTHQGLSSPVTKSFNRGEC

SEQ ID NO: 41 - protein, 5 aa, Artificial Sequence
  DOMAIN (1)..(5): Clone 33 VH CDR1
DTYIQ

SEQ ID NO: 42 - protein, 17 aa, Artificial Sequence
  DOMAIN (1)..(17): Clone 33 VH CDR2
KIDPANGNTMYAQKFQG

SEQ ID NO: 43 - protein, 10 aa, Artificial Sequence
  DOMAIN (1)..(10): Clone 33 VH CDR3
GNLHYALMDY

SEQ ID NO: 44 - protein, 11 aa, Artificial Sequence
  DOMAIN (1)..(11): Clone 33 VL CDR1
KASQTINTYLS

SEQ ID NO: 45 - protein, 7 aa, Artificial Sequence
  DOMAIN (1)..(7): Clone 33 VL CDR2
RANRMPD

SEQ ID NO: 46 - protein, 9 aa, Artificial Sequence
  DOMAIN (1)..(9): Clone 33 VL CDR3
LQYDDFPYT

SEQ ID NO: 47 - protein, 119 aa, Artificial Sequence
  DOMAIN (1)..(119): Clone 33 VH
QVQLVQSGAEVKKPGASVKVSCKASGFNIKDTYIQWVRQAPGQGLEWMGKIDPANGNTMYAQKFQGRVTMTRDTSTSTVYMELSSLRSEDTAVYYCTTGNLHYALMDYWGQGTSVTVSS

SEQ ID NO: 48 - protein, 110 aa, Artificial Sequence
  DOMAIN (1)..(110): Clone 33 VL
DIQMTQSPSSVSASVGDRVTITCKASQTINTYLSWYQQKPGKAPKLLIYRANRMPDGVPSRFSGSGSGTDFTLTISSLQPEDFATYYCLQYDDFPYTFGGGTKLEIKRTV

SEQ ID NO: 49 - protein, 445 aa, Artificial Sequence
  CHAIN (1)..(445): Clone 33 HC
QVQLVQSGAEVKKPGASVKVSCKASGFNIKDTYIQWVRQAPGQGLEWMGKIDPANGNTMYAQKFQGRVTMTRDTSTSTVYMELSSLRSEDTAVYYCTTGNLHYALMDYWGQGTSVTVSSASTKGPSVFPLAPCSRSTSESTAALGCLVKDYFPEPVTVSWNSGALTSGVHTFPAVLQSSGLYSLSSVVTVPSSNFGTQTYTCNVDHKPSNTKVDKTVERKCCVECPPCPAPPVAGPSVFLFPPKPKDTLMISRTPEVTCVVVDVSHEDPEVQFNWYVDGVEVHNAKTKPREEQFNSTFRVVSVLTVVHQDWLNGKEYKCKVSNKGLPAPIEKTISKTKGQPREPQVYTLPPSREEMTKNQVSLTCLVKGFYPSDIAVEWESNGQPENNYKTTPPMLDSDGSFFLYSKLTVDKSRWQQGNVFSCSVMHEALHNHYTQKSLSLSPGK

SEQ ID NO: 50 - protein, 214 aa, Artificial Sequence
  CHAIN (1)..(214): Clone 33 LC
DIQMTQSPSSVSASVGDRVTITCKASQTINTYLSWYQQKPGKAPKLLIYRANRMPDGVPSRFSGSGSGTDFTLTISSLQPEDFATYYCLQYDDFPYTFGGGTKLEIKRTVAAPSVFIFPPSDEQLKSGTASVVCLLNNFYPREAKVQWKVDNALQSGNSQESVTEQDSKDSTYSLSSTLTLSKADYEKHKVYACEVTHQGLSSPVTKSFNRGEC

SEQ ID NO: 51 - protein, 5 aa, Artificial Sequence
  DOMAIN (1)..(5): Clone 35 VH CDR1
DTYIH

SEQ ID NO: 52 - protein, 17 aa, Artificial Sequence
  DOMAIN (1)..(17): Clone 35 VH CDR2
RIDPANGYTEYAQKFQG

SEQ ID NO: 53 - protein, 10 aa, Artificial Sequence
  DOMAIN (1)..(10): Clone 35 VH CDR3
GNLHYALMDY

SEQ ID NO: 54 - protein, 11 aa, Artificial Sequence
  DOMAIN (1)..(11): Clone 35 VL CDR1
KASQAIATYLS

SEQ ID NO: 55 - protein, 7 aa, Artificial Sequence
  DOMAIN (1)..(7): Clone 35 VL CDR2
RANRMVD

SEQ ID NO: 56 - protein, 9 aa, Artificial Sequence
  DOMAIN (1)..(9): Clone 35 VL CDR3
LQFQDFPYT

SEQ ID NO: 57 - protein, 119 aa, Artificial Sequence
  DOMAIN (1)..(119): Clone 35 VH
QVQLVQSGAEVKKPGASVKVSCKASGFNINDTYIHWVRQAPGQGLEWMGRIDPANGYTEYAQKFQGRVTMTRDTSTSTVYMELSSLRSEDTAVYYCTTGNLHYALMDYWGQGTSVTVSS

SEQ ID NO: 58 - protein, 110 aa, Artificial Sequence
  DOMAIN (1)..(110): Clone 35 VL
DIQMTQSPSSVSASVGDRVTITCKASQAIATYLSWYQQKPGKAPKLLIYRANRMVDGVPSRFSGSGSGTDFTLTISSLQPEDFATYYCLQFQDFPYTFGGGTKLEIKRTV

SEQ ID NO: 59 - protein, 445 aa, Artificial Sequence
  CHAIN (1)..(445): Clone 35 HC
QVQLVQSGAEVKKPGASVKVSCKASGFNINDTYIHWVRQAPGQGLEWMGRIDPANGYTEYAQKFQGRVTMTRDTSTSTVYMELSSLRSEDTAVYYCTTGNLHYALMDYWGQGTSVTVSSASTKGPSVFPLAPCSRSTSESTAALGCLVKDYFPEPVTVSWNSGALTSGVHTFPAVLQSSGLYSLSSVVTVPSSNFGTQTYTCNVDHKPSNTKVDKTVERKCCVECPPCPAPPVAGPSVFLFPPKPKDTLMISRTPEVTCVVVDVSHEDPEVQFNWYVDGVEVHNAKTKPREEQFNSTFRVVSVLTVVHQDWLNGKEYKCKVSNKGLPAPIEKTISKTKGQPREPQVYTLPPSREEMTKNQVSLTCLVKGFYPSDIAVEWESNGQPENNYKTTPPMLDSDGSFFLYSKLTVDKSRWQQGNVFSCSVMHEALHNHYTQKSLSLSPGK

SEQ ID NO: 60 - protein, 214 aa, Artificial Sequence
  CHAIN (1)..(214): Clone 35 LC
DIQMTQSPSSVSASVGDRVTITCKASQAIATYLSWYQQKPGKAPKLLIYRANRMVDGVPSRFSGSGSGTDFTLTISSLQPEDFATYYCLQFQDFPYTFGGGTKLEIKRTVAAPSVFIFPPSDEQLKSGTASVVCLLNNFYPREAKVQWKVDNALQSGNSQESVTEQDSKDSTYSLSSTLTLSKADYEKHKVYACEVTHQGLSSPVTKSFNRGEC

SEQ ID NO: 61 - protein, 5 aa, Artificial Sequence
  DOMAIN (1)..(5): Clone 5 VH CDR1
DTYIH

SEQ ID NO: 62 - protein, 17 aa, Artificial Sequence
  DOMAIN (1)..(17): Clone 5 VH CDR2
KIDPANGNTEYAQKFQG

SEQ ID NO: 63 - protein, 10 aa, Artificial Sequence
  DOMAIN (1)..(10): Clone 5 VH CDR3
GNLHYGLMDY

SEQ ID NO: 64 - protein, 11 aa, Artificial Sequence
  DOMAIN (1)..(11): Clone 5 VL CDR1
KASQAINTYHS

SEQ ID NO: 65 - protein, 7 aa, Artificial Sequence
  DOMAIN (1)..(7): Clone 5 VL CDR2
RVNRMVD

SEQ ID NO: 66 - protein, 9 aa, Artificial Sequence
  DOMAIN (1)..(9): Clone 5 VL CDR3
LQYLDFPYT

SEQ ID NO: 67 - protein, 119 aa, Artificial Sequence
  DOMAIN (1)..(119): Clone 5 VH
QVQLVQSGAEVKKPGASVKVSCKASGFNIRDTYIHWVRQAPGQGLEWMGKIDPANGNTEYAQKFQGRVTMTRDTSTSTVYMELSSLRSEDTAVYYCTTGNLHYGLMDYWGQGTSVTVSS

SEQ ID NO: 68 - protein, 110 aa, Artificial Sequence
  DOMAIN (1)..(110): Clone 5 VL
DIQMTQSPSSVSASVGDRVTITCKASQAINTYHSWYQQKPGKAPKLLIYRVNRMVDGVPSRFSGSGSGTDFTLTISSLQPEDFATYYCLQYLDFPYTFGGGTKLEIKRTV

SEQ ID NO: 69 - protein, 445 aa, Artificial Sequence
  CHAIN (1)..(445): Clone 5 HC
QVQLVQSGAEVKKPGASVKVSCKASGFNIRDTYIHWVRQAPGQGLEWMGKIDPANGNTEYAQKFQGRVTMTRDTSTSTVYMELSSLRSEDTAVYYCTTGNLHYGLMDYWGQGTSVTVSSASTKGPSVFPLAPCSRSTSESTAALGCLVKDYFPEPVTVSWNSGALTSGVHTFPAVLQSSGLYSLSSVVTVPSSNFGTQTYTCNVDHKPSNTKVDKTVERKCCVECPPCPAPPVAGPSVFLFPPKPKDTLMISRTPEVTCVVVDVSHEDPEVQFNWYVDGVEVHNAKTKPREEQFNSTFRVVSVLTVVHQDWLNGKEYKCKVSNKGLPAPIEKTISKTKGQPREPQVYTLPPSREEMTKNQVSLTCLVKGFYPSDIAVEWESNGQPENNYKTTPPMLDSDGSFFLYSKLTVDKSRWQQGNVFSCSVMHEALHNHYTQKSLSLSPGK

SEQ ID NO: 70 - protein, 214 aa, Artificial Sequence
  CHAIN (1)..(214): Clone 5 LC
DIQMTQSPSSVSASVGDRVTITCKASQAINTYHSWYQQKPGKAPKLLIYRVNRMVDGVPSRFSGSGSGTDFTLTISSLQPEDFATYYCLQYLDFPYTFGGGTKLEIKRTVAAPSVFIFPPSDEQLKSGTASVVCLLNNFYPREAKVQWKVDNALQSGNSQESVTEQDSKDSTYSLSSTLTLSKADYEKHKVYACEVTHQGLSSPVTKSFNRGEC

SEQ ID NO: 71 - protein, 5 aa, Artificial Sequence
  DOMAIN (1)..(5): Clone 6 VH CDR1
DTYIH

SEQ ID NO: 72 - protein, 17 aa, Artificial Sequence
  DOMAIN (1)..(17): Clone 6 VH CDR2
KIDPANGLTEYAQKFQG

SEQ ID NO: 73 - protein, 10 aa, Artificial Sequence
  DOMAIN (1)..(10): Clone 6 VH CDR3
GNLHYALMDY

SEQ ID NO: 74 - protein, 11 aa, Artificial Sequence
  DOMAIN (1)..(11): Clone 6 VL CDR1
KASQAIATYLS

SEQ ID NO: 75 - protein, 7 aa, Artificial Sequence
  DOMAIN (1)..(7): Clone 6 VL CDR2
RANRMGD

SEQ ID NO: 76 - protein, 9 aa, Artificial Sequence
  DOMAIN (1)..(9): Clone 6 VL CDR3
LQYLDFPYT

SEQ ID NO: 77 - protein, 119 aa, Artificial Sequence
  DOMAIN (1)..(119): Clone 6 VH
QVQLVQSGAEVKKPGASVKVSCKASGFNICDTYIHWVRQAPGQGLEWMGKIDPANGLTEYAQKFQGRVTMTRDTSTSTVYMELSSLRSEDTAVYYCTTGNLHYALMDYWGQGTSVTVSS

SEQ ID NO: 78 - protein, 110 aa, Artificial Sequence
  DOMAIN (1)..(110): Clone 6 VL
DIQMTQSPSSVSASVGDRVTITCKASQAIATYLSWYQQKPGKAPKLLIYRANRMGDGVPSRFSGSGSGTDFTLTISSLLPEDFATYYCLQYLDFPYTFGGGTKLEIKRTV

SEQ ID NO: 79 - protein, 445 aa, Artificial Sequence
  CHAIN (1)..(445): Clone 6 HC
QVQLVQSGAEVKKPGASVKVSCKASGFNICDTYIHWVRQAPGQGLEWMGKIDPANGLTEYAQKFQGRVTMTRDTSTSTVYMELSSLRSEDTAVYYCTTGNLHYALMDYWGQGTSVTVSSASTKGPSVFPLAPCSRSTSESTAALGCLVKDYFPEPVTVSWNSGALTSGVHTFPAVLQSSGLYSLSSVVTVPSSNFGTQTYTCNVDHKPSNTKVDKTVERKCCVECPPCPAPPVAGPSVFLFPPKPKDTLMISRTPEVTCVVVDVSHEDPEVQFNWYVDGVEVHNAKTKPREEQFNSTFRVVSVLTVVHQDWLNGKEYKCKVSNKGLPAPIEKTISKTKGQPREPQVYTLPPSREEMTKNQVSLTCLVKGFYPSDIAVEWESNGQPENNYKTTPPMLDSDGSFFLYSKLTVDKSRWQQGNVFSCSVMHEALHNHYTQKSLSLSPGK

SEQ ID NO: 80 - protein, 214 aa, Artificial Sequence
  CHAIN (1)..(214): Clone 6 LC
DIQMTQSPSSVSASVGDRVTITCKASQAIATYLSWYQQKPGKAPKLLIYRANRMGDGVPSRFSGSGSGTDFTLTISSLLPEDFATYYCLQYLDFPYTFGGGTKLEIKRTVAAPSVFIFPPSDEQLKSGTASVVCLLNNFYPREAKVQWKVDNALQSGNSQESVTEQDSKDSTYSLSSTLTLSKADYEKHKVYACEVTHQGLSSPVTKSFNRGEC

SEQ ID NO: 81 - protein, 5 aa, Artificial Sequence
  DOMAIN (1)..(5): Clone 17 VH CDR1
DTYIH

SEQ ID NO: 82 - protein, 17 aa, Artificial Sequence
  DOMAIN (1)..(17): Clone 17 VH CDR2
KIDPANGQTEYAQKFQG

SEQ ID NO: 83 - protein, 10 aa, Artificial Sequence
  DOMAIN (1)..(10): Clone 17 VH CDR3
GNLHYALMDY

SEQ ID NO: 84 - protein, 11 aa, Artificial Sequence
  DOMAIN (1)..(11): Clone 17 VL CDR1
KASQATNTYLS

SEQ ID NO: 85 - protein, 7 aa, Artificial Sequence
  DOMAIN (1)..(7): Clone 17 VL CDR2
RVNRVVD

SEQ ID NO: 86 - protein, 9 aa, Artificial Sequence
  DOMAIN (1)..(9): Clone 17 VL CDR3
LQYRDFPYT

SEQ ID NO: 87 - protein, 119 aa, Artificial Sequence
  DOMAIN (1)..(119): Clone 17 VH
QVQLVQSGAEVKKPGASVKVSCKASGFCIKDTYIHWVRQAPGQGLEWMGKIDPANGQTEYAQKFQGRVTMTRDTSTSTVYMELSSLRSEDTAVYYCTTGNLHYALMDYWGQGTSVTVSS

SEQ ID NO: 88 - protein, 110 aa, Artificial Sequence
  DOMAIN (1)..(110): Clone 17 VL
DIQMTQSPSSVSASVGDRVTITCKASQATNTYLSWYQQKPGKAPKLLIYRVNRVVDGVPSRFSGSGSGTDFTLTISSLQPEDFATYYCLQYRDFPYTFGGGTKLEIKRTV

SEQ ID NO: 89 - protein, 445 aa, Artificial Sequence
  CHAIN (1)..(445): Clone 17 HC
QVQLVQSGAEVKKPGASVKVSCKASGFCIKDTYIHWVRQAPGQGLEWMGKIDPANGQTEYAQKFQGRVTMTRDTSTSTVYMELSSLRSEDTAVYYCTTGNLHYALMDYWGQGTSVTVSSASTKGPSVFPLAPCSRSTSESTAALGCLVKDYFPEPVTVSWNSGALTSGVHTFPAVLQSSGLYSLSSVVTVPSSNFGTQTYTCNVDHKPSNTKVDKTVERKCCVECPPCPAPPVAGPSVFLFPPKPKDTLMISRTPEVTCVVVDVSHEDPEVQFNWYVDGVEVHNAKTKPREEQFNSTFRVVSVLTVVHQDWLNGKEYKCKVSNKGLPAPIEKTISKTKGQPREPQVYTLPPSREEMTKNQVSLTCLVKGFYPSDIAVEWESNGQPENNYKTTPPMLDSDGSFFLYSKLTVDKSRWQQGNVFSCSVMHEALHNHYTQKSLSLSPGK

SEQ ID NO: 90 - protein, 214 aa, Artificial Sequence
  CHAIN (1)..(214): Clone 17 LC
DIQMTQSPSSVSASVGDRVTITCKASQATNTYLSWYQQKPGKAPKLLIYRVNRVVDGVPSRFSGSGSGTDFTLTISSLQPEDFATYYCLQYRDFPYTFGGGTKLEIKRTVAAPSVFIFPPSDEQLKSGTASVVCLLNNFYPREAKVQWKVDNALQSGNSQESVTEQDSKDSTYSLSSTLTLSKADYEKHKVYACEVTHQGLSSPVTKSFNRGEC

SEQ ID NO: 91 - protein, 5 aa, Artificial Sequence
  DOMAIN (1)..(5): Clone 18 VH CDR1
DTYIH

SEQ ID NO: 92 - protein, 17 aa, Artificial Sequence
  DOMAIN (1)..(17): Clone 18 VH CDR2
KIDPANGMTEYAQKFQG

SEQ ID NO: 93 - protein, 10 aa, Artificial Sequence
  DOMAIN (1)..(10): Clone 18 VH CDR3
GNLHYALMDY

SEQ ID NO: 94 - protein, 11 aa, Artificial Sequence
  DOMAIN (1)..(11): Clone 18 VL CDR1
KASQAPNTYLS

SEQ ID NO: 95 - protein, 7 aa, Artificial Sequence
  DOMAIN (1)..(7): Clone 18 VL CDR2
RANRMVD

SEQ ID NO: 96 - protein, 9 aa, Artificial Sequence
  DOMAIN (1)..(9): Clone 18 VL CDR3
LQYEDFPYT

SEQ ID NO: 97 - protein, 119 aa, Artificial Sequence
  DOMAIN (1)..(119): Clone 18 VH
QVQLVQSGAEVKKPGASVKVSCQASGFNIKDTYIHWVRQAPGQGLGWMGKIDPANGMTEYAQKFQGRVTVTRDTSTSTVYMELSSLRSEDTAVYYCTTGNLHYALMDYWGQGTSVTVSS

SEQ ID NO: 98 - protein, 110 aa, Artificial Sequence
  DOMAIN (1)..(110): Clone 18 VL
DIQMTQSPSSVSASVGDRVTITCKASQAPNTYLSWYQQKPGKAPKLLIYRANRMVDGVPSRFSGSGSGTDFTLTISSLQPEDFATYYCLQYEDFPYTFGGGTKLEIKRTV

SEQ ID NO: 99 - protein, 445 aa, Artificial Sequence
  CHAIN (1)..(445): Clone 18 HC
QVQLVQSGAEVKKPGASVKVSCQASGFNIKDTYIHWVRQAPGQGLGWMGKIDPANGMTEYAQKFQGRVTVTRDTSTSTVYMELSSLRSEDTAVYYCTTGNLHYALMDYWGQGTSVTVSSASTKGPSVFPLAPCSRSTSESTAALGCLVKDYFPEPVTVSWNSGALTSGVHTFPAVLQSSGLYSLSSVVTVPSSNFGTQTYTCNVDHKPSNTKVDKTVERKCCVECPPCPAPPVAGPSVFLFPPKPKDTLMISRTPEVTCVVVDVSHEDPEVQFNWYVDGVEVHNAKTKPREEQFNSTFRVVSVLTVVHQDWLNGKEYKCKVSNKGLPAPIEKTISKTKGQPREPQVYTLPPSREEMTKNQVSLTCLVKGFYPSDIAVEWESNGQPENNYKTTPPMLDSDGSFFLYSKLTVDKSRWQQGNVFSCSVMHEALHNHYTQKSLSLSPGK

SEQ ID NO: 100 - protein, 214 aa, Artificial Sequence
  CHAIN (1)..(214): Clone 18 LC
DIQMTQSPSSVSASVGDRVTITCKASQAPNTYLSWYQQKPGKAPKLLIYRANRMVDGVPSRFSGSGSGTDFTLTISSLQPEDFATYYCLQYEDFPYTFGGGTKLEIKRTVAAPSVFIFPPSDEQLKSGTASVVCLLNNFYPREAKVQWKVDNALQSGNSQESVTEQDSKDSTYSLSSTLTLSKADYEKHKVYACEVTHQGLSSPVTKSFNRGEC

SEQ ID NO: 101 - protein, 5 aa, Artificial Sequence
  DOMAIN (1)..(5): Clone 19 VH CDR1
DTYIH

SEQ ID NO: 102 - protein, 17 aa, Artificial Sequence
  DOMAIN (1)..(17): Clone 19 VH CDR2
KIDPANGATEYAQKFQG

SEQ ID NO: 103 - protein, 10 aa, Artificial Sequence
  DOMAIN (1)..(10): Clone 19 VH CDR3
GNLHYGLMDY

SEQ ID NO: 104 - protein, 11 aa, Artificial Sequence
  DOMAIN (1)..(11): Clone 19 VL CDR1
KASQAINTYLS

SEQ ID NO: 105 - protein, 7 aa, Artificial Sequence
  DOMAIN (1)..(7): Clone 19 VL CDR2
RANRMGD

SEQ ID NO: 106 - protein, 9 aa, Artificial Sequence
  DOMAIN (1)..(9): Clone 19 VL CDR3
LQSDDFPYT

SEQ ID NO: 107 - protein, 119 aa, Artificial Sequence
  DOMAIN (1)..(119): Clone 19 VH
QVQLVQSGAEVKKPGASVKVSCKASGFNMKDTYIHWVRQAPGQGLEWMGKIDPANGATEYAQKFQGRVTMTRDTSTSTVYMELSSLRSEDTAVYYCTTGNLHYGLMDYWGQGTSVTVSS

SEQ ID NO: 108 - protein, 110 aa, Artificial Sequence
  DOMAIN (1)..(110): Clone 19 VL
DIQMTQSPSSVSASVGDRVTITCKASQAINTYLSWYQQKPGKAPKLLIYRANRMGDGVPSRFSGSGSGTDFTLTISSLQPEDFATYYCLQSDDFPYTFGGGTKLEIKRTV

SEQ ID NO: 109 - protein, 445 aa, Artificial Sequence
  CHAIN (1)..(445): Clone 19 HC
QVQLVQSGAEVKKPGASVKVSCKASGFNMKDTYIHWVRQAPGQGLEWMGKIDPANGATEYAQKFQGRVTMTRDTSTSTVYMELSSLRSEDTAVYYCTTGNLHYGLMDYWGQGTSVTVSSASTKGPSVFPLAPCSRSTSESTAALGCLVKDYFPEPVTVSWNSGALTSGVHTFPAVLQSSGLYSLSSVVTVPSSNFGTQTYTCNVDHKPSNTKVDKTVERKCCVECPPCPAPPVAGPSVFLFPPKPKDTLMISRTPEVTCVVVDVSHEDPEVQFNWYVDGVEVHNAKTKPREEQFNSTFRVVSVLTVVHQDWLNGKEYKCKVSNKGLPAPIEKTISKTKGQPREPQVYTLPPSREEMTKNQVSLTCLVKGFYPSDIAVEWESNGQPENNYKTTPPMLDSDGSFFLYSKLTVDKSRWQQGNVFSCSVMHEALHNHYTQKSLSLSPGK

SEQ ID NO: 110 - protein, 214 aa, Artificial Sequence
  DOMAIN (1)..(214): Clone 19 LC
DIQMTQSPSSVSASVGDRVTITCKASQAINTYLSWYQQKPGKAPKLLIYRANRMGDGVPSRFSGSGSGTDFTLTISSLQPEDFATYYCLQSDDFPYTFGGGTKLEIKRTVAAPSVFIFPPSDEQLKSGTASVVCLLNNFYPREAKVQWKVDNALQSGNSQESVTEQDSKDSTYSLSSTLTLSKADYEKHKVYACEVTHQGLSSPVTKSFNRGEC

SEQ ID NO: 111 - protein, 5 aa, Artificial Sequence
  DOMAIN (1)..(5): Clone 20 VH CDR1
DTYIH

SEQ ID NO: 112 - protein, 17 aa, Artificial Sequence
  DOMAIN (1)..(17): Clone 20 VH CDR2
KIDPANGDTEYAQKFQG

SEQ ID NO: 113 - protein, 10 aa, Artificial Sequence
  DOMAIN (1)..(10): Clone 20 VH CDR3
GNLHYALMDY

SEQ ID NO: 114 - protein, 11 aa, Artificial Sequence
  DOMAIN (1)..(11): Clone 20 VL CDR1
KASQAINTYLS

SEQ ID NO: 115 - protein, 7 aa, Artificial Sequence
  DOMAIN (1)..(7): Clone 20 VL CDR2
RANRAVD

SEQ ID NO: 116 - protein, 9 aa, Artificial Sequence
  DOMAIN (1)..(9): Clone 20 VL CDR3
LQYLDFPYT

SEQ ID NO: 117 - protein, 119 aa, Artificial Sequence
  DOMAIN (1)..(119): Clone 20 VH
QVQLVQSGAEVKKPGASVKVSCKASGFNMKDTYIHWVRQAPGQGLEWMGKIDPANGDTEYAQKFQGRVTMTRDTSTSTVYMELSSLRSEDTAVYYCTTGNLHYALMDYWGQGTSVTVSS

SEQ ID NO: 118 - protein, 110 aa, Artificial Sequence
  DOMAIN (1)..(110): Clone 20 VL
DIQMTQSPSSVSASVGDRVTITCKASQAINTYLSWYQQKPGKAPKLLIYRANRAVDGVPSRFSGSGSGTDFTLTISSLQPEDFATYYCLQYLDFPYTFGGGTKLEIKRTV

SEQ ID NO: 119 - protein, 445 aa, Artificial Sequence
  CHAIN (1)..(445): Clone 20 HC
QVQLVQSGAEVKKPGASVKVSCKASGFNMKDTYIHWVRQAPGQGLEWMGKIDPANGDTEYAQKFQGRVTMTRDTSTSTVYMELSSLRSEDTAVYYCTTGNLHYALMDYWGQGTSVTVSSASTKGPSVFPLAPCSRSTSESTAALGCLVKDYFPEPVTVSWNSGALTSGVHTFPAVLQSSGLYSLSSVVTVPSSNFGTQTYTCNVDHKPSNTKVDKTVERKCCVECPPCPAPPVAGPSVFLFPPKPKDTLMISRTPEVTCVVVDVSHEDPEVQFNWYVDGVEVHNAKTKPREEQFNSTFRVVSVLTVVHQDWLNGKEYKCKVSNKGLPAPIEKTISKTKGQPREPQVYTLPPSREEMTKNQVSLTCLVKGFYPSDIAVEWESNGQPENNYKTTPPMLDSDGSFFLYSKLTVDKSRWQQGNVFSCSVMHEALHNHYTQKSLSLSPGK

SEQ ID NO: 120 - protein, 214 aa, Artificial Sequence
  CHAIN (1)..(214): Clone 20 LC
DIQMTQSPSSVSASVGDRVTITCKASQAINTYLSWYQQKPGKAPKLLIYRANRAVDGVPSRFSGSGSGTDFTLTISSLQPEDFATYYCLQYLDFPYTFGGGTKLEIKRTVAAPSVFIFPPSDEQLKSGTASVVCLLNNFYPREAKVQWKVDNALQSGNSQESVTEQDSKDSTYSLSSTLTLSKADYEKHKVYACEVTHQGLSSPVTKSFNRGEC

SEQ ID NO: 121 - protein, 5 aa, Artificial Sequence
  DOMAIN (1)..(5): Clone 2-9 VH CDR1
DTYIH

SEQ ID NO: 122 - protein, 17 aa, Artificial Sequence
  DOMAIN (1)..(17): Clone 2-9 VH CDR2
RIDPANGNSEYAQKFQG

SEQ ID NO: 123 - protein, 10 aa, Artificial Sequence
  DOMAIN (1)..(10): Clone 2-9 VH CDR3
GNLHYALMDY

SEQ ID NO: 124 - protein, 11 aa, Artificial Sequence
  DOMAIN (1)..(11): Clone 2-9 VL CDR1
KASQPINTYLS

SEQ ID NO: 125 - protein, 7 aa, Artificial Sequence
  DOMAIN (1)..(7): Clone 2-9 VL CDR2
RVNRKVD

SEQ ID NO: 126 - protein, 9 aa, Artificial Sequence
  DOMAIN (1)..(9): Clone 2-9 VL CDR3
LQYLDFPYT

SEQ ID NO: 127 - protein, 119 aa, Artificial Sequence
  DOMAIN (1)..(119): Clone 2-9 VH
QVQLVQSGAEVKKPGASVKASCKASGFNIQDTYIHWVRQAPGQGLEWMGRIDPANGNSEYAQKFQGRVTMTRDTSTSTVYMELSSLRSEDTAVYYCTTGNLHYALMDYWGQGTSVTVSS

SEQ ID NO: 128 - protein, 110 aa, Artificial Sequence
  DOMAIN (1)..(110): Clone 2-9 VL
DIQMTQSPSSVSASVGDRVTITCKASQPINTYLSWYQQKPGKAPKLLIYRVNRKVDGVPSRFSGSGSGTDFTLTISSLQPEDFATYYCLQYLDFPYTFGGGTKLEIKRTV

SEQ ID NO: 129 - protein, 445 aa, Artificial Sequence
  CHAIN (1)..(445): Clone 2-9 HC
QVQLVQSGAEVKKPGASVKASCKASGFNIQDTYIHWVRQAPGQGLEWMGRIDPANGNSEYAQKFQGRVTMTRDTSTSTVYMELSSLRSEDTAVYYCTTGNLHYALMDYWGQGTSVTVSSASTKGPSVFPLAPCSRSTSESTAALGCLVKDYFPEPVTVSWNSGALTSGVHTFPAVLQSSGLYSLSSVVTVPSSNFGTQTYTCNVDHKPSNTKVDKTVERKCCVECPPCPAPPVAGPSVFLFPPKPKDTLMISRTPEVTCVVVDVSHEDPEVQFNWYVDGVEVHNAKTKPREEQFNSTFRVVSVLTVVHQDWLNGKEYKCKVSNKGLPAPIEKTISKTKGQPREPQVYTLPPSREEMTKNQVSLTCLVKGFYPSDIAVEWESNGQPENNYKTTPPMLDSDGSFFLYSKLTVDKSRWQQGNVFSCSVMHEALHNHYTQKSLSLSPGK

SEQ ID NO: 130 - protein, 214 aa, Artificial Sequence
  CHAIN (1)..(214): Clone 2-9 LC
DIQMTQSPSSVSASVGDRVTITCKASQPINTYLSWYQQKPGKAPKLLIYRVNRKVDGVPSRFSGSGSGTDFTLTISSLQPEDFATYYCLQYLDFPYTFGGGTKLEIKRTVAAPSVFIFPPSDEQLKSGTASVVCLLNNFYPREAKVQWKVDNALQSGNSQESVTEQDSKDSTYSLSSTLTLSKADYEKHKVYACEVTHQGLSSPVTKSFNRGEC

SEQ ID NO: 131 - protein, 5 aa, Artificial Sequence
  DOMAIN (1)..(5): Clone 2-11 VH CDR1
DTYIH

SEQ ID NO: 132 - protein, 17 aa, Artificial Sequence
  DOMAIN (1)..(17): Clone 2-11 VH CDR2
KIDPANGGTEYAQKFQG

SEQ ID NO: 133 - protein, 10 aa, Artificial Sequence
  DOMAIN (1)..(10): Clone 2-11 VH CDR3
GNLHYALMDY

SEQ ID NO: 134 - protein, 11 aa, Artificial Sequence
  DOMAIN (1)..(11): Clone 2-11 VL CDR1
KASQPINTYLS

SEQ ID NO: 135 - protein, 7 aa, Artificial Sequence
  DOMAIN (1)..(7): Clone 2-11 VL CDR2
RVNRKVD

SEQ ID NO: 136 - protein, 9 aa, Artificial Sequence
  DOMAIN (1)..(9): Clone 2-11 VL CDR3
LQYVDFPYT

SEQ ID NO: 137 - protein, 119 aa, Artificial Sequence
  DOMAIN (1)..(119): Clone 2-11 VH
QVQLVQSGAEVKKPGASVKVSCKASGFNIKDTYIHWVRQAPGQGLEWMGKIDPANGGTEYAQKFQGRVTMTRDTSTSTVYMELSSLRSEDTAVYYCTTGNLHYALMDYWGQGTSVTVSS

SEQ ID NO: 138 - protein, 110 aa, Artificial Sequence
  DOMAIN (1)..(110): Clone 2-11 VL
DIQMTQSPSSVSASVGDRVTITCKASQPINTYLSWYQQKPGKAPKLLIYRVNRKVDGVPSRFSGSGSGTDFTLTISSLQPEDFATYYCLQYVDFPYTFGGGTKLEIKRTV

SEQ ID NO: 139 - protein, 445 aa, Artificial Sequence
  CHAIN (1)..(445): Clone 2-11 HC
QVQLVQSGAEVKKPGASVKVSCKASGFNIKDTYIHWVRQAPGQGLEWMGKIDPANGGTEYAQKFQGRVTMTRDTSTSTVYMELSSLRSEDTAVYYCTTGNLHYALMDYWGQGTSVTVSSASTKGPSVFPLAPCSRSTSESTAALGCLVKDYFPEPVTVSWNSGALTSGVHTFPAVLQSSGLYSLSSVVTVPSSNFGTQTYTCNVDHKPSNTKVDKTVERKCCVECPPCPAPPVAGPSVFLFPPKPKDTLMISRTPEVTCVVVDVSHEDPEVQFNWYVDGVEVHNAKTKPREEQFNSTFRVVSVLTVVHQDWLNGKEYKCKVSNKGLPAPIEKTISKTKGQPREPQVYTLPPSREEMTKNQVSLTCLVKGFYPSDIAVEWESNGQPENNYKTTPPMLDSDGSFFLYSKLTVDKSRWQQGNVFSCSVMHEALHNHYTQKSLSLSPGK

SEQ ID NO: 140 - protein, 214 aa, Artificial Sequence
  CHAIN (1)..(214): Clone 2-11 LC
DIQMTQSPSSVSASVGDRVTITCKASQPINTYLSWYQQKPGKAPKLLIYRVNRKVDGVPSRFSGSGSGTDFTLTISSLQPEDFATYYCLQYVDFPYTFGGGTKLEIKRTVAAPSVFIFPPSDEQLKSGTASVVCLLNNFYPREAKVQWKVDNALQSGNSQESVTEQDSKDSTYSLSSTLTLSKADYEKHKVYACEVTHQGLSSPVTKSFNRGEC

SEQ ID NO: 141 - protein, 5 aa, Artificial Sequence
  DOMAIN (1)..(5): Consensus VH CDR1
DTYIH

SEQ ID NO: 142 - protein, 17 aa, Artificial Sequence
  DOMAIN (1)..(17): Consensus VH CDR2
  UNSURE (1)..(1): The 'Xaa' at location 1 stands for any amino acid
  UNSURE (8)..(8): The 'Xaa' at location 8 stands for any amino acid
XIDPANGXTEYAQKFQG

SEQ ID NO: 143 - protein, 10 aa, Artificial Sequence
  DOMAIN (1)..(10): Consensus VH CDR3
  UNSURE (6)..(6): The 'Xaa' at location 6 stands for any amino acid
GNLHYXLMDY

SEQ ID NO: 144 - protein, 11 aa, Artificial Sequence
  DOMAIN (1)..(11): Consensus VL CDR1
  UNSURE (5)..(5): The 'Xaa' at location 5 stands for any amino acid
  UNSURE (6)..(6): The 'Xaa' at location 6 stands for any amino acid
  UNSURE (7)..(7): The 'Xaa' at location 7 stands for any amino acid
  UNSURE (10)..(10): The 'Xaa' at location 10 stands for any amino acid
KASQXXXTYXS

SEQ ID NO: 145 - protein, 7 aa, Artificial Sequence
  DOMAIN (1)..(7): Consensus VL CDR2
  UNSURE (2)..(2): The 'Xaa' at location 2 stands for any amino acid
  UNSURE (5)..(5): The 'Xaa' at location 5 stands for any amino acid
  UNSURE (6)..(6): The 'Xaa' at location 6 stands for any amino acid
RXNRXXD

SEQ ID NO: 146 - protein, 9 aa, Artificial Sequence
  DOMAIN (1)..(9): Consensus VL CDR3
  UNSURE (4)..(4): The 'Xaa' at location 4 stands for any amino acid
LQYXDFPYT

SEQ ID NO: 147 - protein, 119 aa, Artificial Sequence
  DOMAIN (1)..(119): Consensus VH
  UNSURE (28)..(28): The 'Xaa' at location 28 stands for any amino acid
  UNSURE (29)..(29): The 'Xaa' at location 29 stands for any amino acid
  UNSURE (30)..(30): The 'Xaa' at location 30 stands for any amino acid
  UNSURE (50)..(50): The 'Xaa' at location 50 stands for any amino acid
  UNSURE (57)..(57): The 'Xaa' at location 57 stands for any amino acid
  UNSURE (104)..(104): The 'Xaa' at location 104 stands for any amino acid
QVQLVQSGAEVKKPGASVKVSCKASGFXXXDTYIHWVRQAPGQGLEWMGXIDPANGXTEYAQKFQGRVTMTRDTSTSTVYMELSSLRSEDTAVYYCTTGNLHYXLMDYWGQGTSVTVSS

SEQ ID NO: 148 - protein, 110 aa, Artificial Sequence
  DOMAIN (1)..(110): Consensus VL
  UNSURE (28)..(28): The 'Xaa' at location 28 stands for any amino acid
  UNSURE (29)..(29): The 'Xaa' at location 29 stands for any amino acid
  UNSURE (30)..(30): The 'Xaa' at location 30 stands for any amino acid
  UNSURE (33)..(33): The 'Xaa' at location 33 stands for any amino acid
  UNSURE (51)..(51): The 'Xaa' at location 51 stands for any amino acid
  UNSURE (54)..(54): The 'Xaa' at location 54 stands for any amino acid
  UNSURE (55)..(55): The 'Xaa' at location 55 stands for any amino acid
  UNSURE (92)..(92): The 'Xaa' at location 92 stands for any amino acid
DIQMTQSPSSVSASVGDRVTITCKASQXXXTYXSWYQQKPGKAPKLLIYRXNRXXDGVPSRFSGSGSGTDFTLTISSLQPEDFATYYCLQYXDFPYTFGGGTKLEIKRTV

SEQ ID NO: 149 - protein, 445 aa, Artificial Sequence
  CHAIN (1)..(445): Consensus HC
  UNSURE (28)..(28): The 'Xaa' at location 28 stands for any amino acid
  UNSURE (29)..(29): The 'Xaa' at location 29 stands for any amino acid
  UNSURE (30)..(30): The 'Xaa' at location 30 stands for any amino acid
  UNSURE (57)..(57): The 'Xaa' at location 57 stands for any amino acid
  UNSURE (104)..(104): The 'Xaa' at location 104 stands for any amino acid
QVQLVQSGAEVKKPGASVKVSCKASGFXXXDTYIHWVRQAPGQGLEWMGKIDPANGXTEYAQKFQGRVTMTRDTSTSTVYMELSSLRSEDTAVYYCTTGNLHYXLMDYWGQGTSVTVSSASTKGPSVFPLAPCSRSTSESTAALGCLVKDYFPEPVTVSWNSGALTSGVHTFPAVLQSSGLYSLSSVVTVPSSNFGTQTYTCNVDHKPSNTKVDKTVERKCCVECPPCPAPPVAGPSVFLFPPKPKDTLMISRTPEVTCVVVDVSHEDPEVQFNWYVDGVEVHNAKTKPREEQFNSTFRVVSVLTVVHQDWLNGKEYKCKVSNKGLPAPIEKTISKTKGQPREPQVYTLPPSREEMTKNQVSLTCLVKGFYPSDIAVEWESNGQPENNYKTTPPMLDSDGSFFLYSKLTVDKSRWQQGNVFSCSVMHEALHNHYTQKSLSLSPGK

SEQ ID NO: 150 - protein, 214 aa, Artificial Sequence
  CHAIN (1)..(214): Consensus LC
  UNSURE (28)..(28): The 'Xaa' at location 28 stands for any amino acid
  UNSURE (29)..(29): The 'Xaa' at location 29 stands for any amino acid
  UNSURE (30)..(30): The 'Xaa' at location 30 stands for any amino acid
  UNSURE (33)..(33): The 'Xaa' at location 33 stands for any amino acid
  UNSURE (51)..(51): The 'Xaa' at location 51 stands for any amino acid
  UNSURE (54)..(54): The 'Xaa' at location 54 stands for any amino acid
  UNSURE (55)..(55): The 'Xaa' at location 55 stands for any amino acid
  UNSURE (92)..(92): The 'Xaa' at location 92 stands for any amino acid
DIQMTQSPSSVSASVGDRVTITCKASQXXXTYXSWYQQKPGKAPKLLIYRXNRXXDGVPSRFSGSGSGTDFTLTISSLQPEDFATYYCLQYXDFPYTFGGGTKLEIKRTVAAPSVFIFPPSDEQLKSGTASVVCLLNNFYPREAKVQWKVDNALQSGNSQESVTEQDSKDSTYSLSSTLTLSKADYEKHKVYACEVTHQGLSSPVTKSFNRGEC

SEQ ID NO: 151 - protein, 5 aa, Artificial Sequence
  DOMAIN (1)..(5): 29.39/44.21 VH CDR1
DTYIH

SEQ ID NO: 152 - protein, 5 aa, Artificial Sequence
  DOMAIN (1)..(5): 3.10 VH CDR1
TYDVS

SEQ ID NO: 153 - protein, 5 aa, Artificial Sequence
  DOMAIN (1)..(5): 30.19/6.62 VH CDR1
DYSIH

SEQ ID NO: 154 - protein, 17 aa, Artificial Sequence
  DOMAIN (1)..(17): 29.39/44.21 VH CDR2
KIDPANGNTEYDLNFQG

SEQ ID NO: 155 - protein, 16 aa, Artificial Sequence
  DOMAIN (1)..(16): 3.10 VH CDR2
VIWTGGGTNYNSTFMS

SEQ ID NO: 156 - protein, 17 aa, Artificial Sequence
  DOMAIN (1)..(17): 30.19/6.62 VH CDR2
WMNTETGEPAYADDFKG

SEQ ID NO: 157 - protein, 10 aa, Artificial Sequence
  DOMAIN (1)..(10): 29.39/44.21 VH CDR3
GNLHYYLMDY

SEQ ID NO: 158 - protein, 3 aa, Artificial Sequence
  DOMAIN (1)..(3): 3.10 VH CDR3
VDY

SEQ ID NO: 159 - protein, 8 aa, Artificial Sequence
  DOMAIN (1)..(8): 30.19/6.62 VH CDR3
SSYGYFDY

SEQ ID NO: 160 - protein, 11 aa, Artificial Sequence
  DOMAIN (1)..(11): 29.39/30.19 VL CDR1
KASQAINTYLS

SEQ ID NO: 161 - protein, 16 aa, Artificial Sequence
  DOMAIN (1)..(16): 6.62 VL CDR1
RSSQTLEHINGNTYLE

SEQ ID NO: 162 - protein, 16 aa, Artificial Sequence
  DOMAIN (1)..(16): 44.21 VL CDR1
RSSQSLVHSNGNTYLH

SEQ ID NO: 163 - protein, 16 aa, Artificial Sequence
  DOMAIN (1)..(16): 3.10 VL CDR1
RSSQSLVHNNGNTYLH

SEQ ID NO: 164 - protein, 7 aa, Artificial Sequence
  DOMAIN (1)..(7): 29.39/30.19 VL CDR2
RANRMVD

SEQ ID NO: 165 - protein, 7 aa, Artificial Sequence
  DOMAIN (1)..(7): 6.62 VL CDR2
KVSDRFS

SEQ ID NO: 166 - protein, 7 aa, Artificial Sequence
  DOMAIN (1)..(7): 44.21/3.10 VL CDR2
KVSNRFS

SEQ ID NO: 167 - protein, 9 aa, Artificial Sequence
  DOMAIN (1)..(9): 29.39/30.19 VL CDR3
LQYDDFPYT

SEQ ID NO: 168 - protein, 9 aa, Artificial Sequence
  DOMAIN (1)..(9): 6.62 VL CDR3
FQGSHFPLT

SEQ ID NO: 169 - protein, 9 aa, Artificial Sequence
  DOMAIN (1)..(9): 44.21/3.10 VL CDR3
SQNAHVPWT

SEQ ID NO: 170 - protein, 119 aa, Artificial Sequence
  DOMAIN (1)..(119): 29.39/44.21 VH
EVKLMESGAELVKPGASVKLSCTASGFNIKDTYIHWVKQRPEQGLEWIGKIDPANGNTEYDLNFQGRATITADTSSNTAYLQLSSLTSEDTAVYYCTTGNLHYYLMDYWGQGTSVTSLE

SEQ ID NO: 171 - protein, 117 aa, Artificial Sequence
  DOMAIN (1)..(117): 30.19/6.62 VH
QIQLVQSGPELKKPGETVKISCKASGYSFTDYSIHWVKQAPGKGLKWMGWMNTETGEPAYADDFKGRFAFSLETAASTAYLQINHLRDEDTATYFCTRSSYGYFDYWGQGTTLTVSS

SEQ ID NO: 172 - protein, 111 aa, Artificial Sequence
  DOMAIN (1)..(111): 3.10 VH
EVQLVESGPGLVAPSQSLSITCTVSGFSLTTYDVSWIRQPPGKGLEWLGVIWTGGGTNYNSTFMSRLTISKDNSKNQVFLKMNSLQTDDTATYYCVRVDYWGQGTTLTVSR

SEQ ID NO: 173 - protein, 108 aa, Artificial Sequence
  DOMAIN (1)..(108): 29.39/30.19 VL
DIVMTQSPSSMYASLGERVTITCKASQAINTYLSWFQQKPGKSPKTLIYRANRMVDGVPSRFSGSGSGQDYSLTISSLDYEDMGIYYCLQYDDFPYTFGGGTKLEIKR

SEQ ID NO: 174 - protein, 112 aa, Artificial Sequence
  DOMAIN (1)..(112): 6.62 VL
DVVMTQTPLSLPVSLGDQAAISCRSSQTLEHINGNTYLEWYLQKPGQSPKLLIYKVSDRFSGVPDRFSGSGSGTGFTLKISRVEAEDLGVYYCFQGSHFPLTFGGGTKLELK

SEQ ID NO: 175 - protein, 113 aa, Artificial Sequence
  DOMAIN (1)..(113): 3.10 VL
DVVMTQTPLSLPVSLGGHASISCRSSQSLVHNNGNTYLHWFLQKPGQSPKLLIYKVSNRFSGVPDRFSGSGSGTDFTLKISRVEAEDLGVYFCSQNAHVPWTFGGGTKLEIKR

SEQ ID NO: 176 - protein, 113 aa, Artificial Sequence
  DOMAIN (1)..(113): 44.21 VL
DIVMTQTPLSLPVSLGDHASISCRSSQSLVHSNGNTYLHWFLQKPGQSPKLLIYKVSNRFSGVPDRFSGSGSGTDFTLKISRVEAEDLGVYFCSQNAHVPWTFGGGTKRKSNE

SEQ ID NO: 177 - protein, 10 aa, Artificial Sequence
  DOMAIN (1)..(10): Consensus humanized 29.39 VH CDR1 GFX1X2X3DTYI X4 wherein X1=N or C; X2=I, P, L or M; X3=K, N, R, C or Q; X4=H or Q
  UNSURE (3)..(3): The 'Xaa' at location 3 stands for Asn or Cys
  UNSURE (4)..(4): The 'Xaa' at location 4 stands for Ile, Pro, Leu or Met
  UNSURE (5)..(5): The 'Xaa' at location 5 stands for Lys, Asn, Arg, Cys or Gln
  UNSURE (10)..(10): The 'Xaa' at location 10 stands for His or Gln
GFXXXDTYIX

SEQ ID NO: 178 - protein, 10 aa, Artificial Sequence
  DOMAIN (1)..(10): Consensus humanized 29.39 VH CDR2 X1IDPANGX2X3X4 wherein X1=K or R; X2=N, G, F, Y, A, D, L, M or Q; X3=S or T; X4=E or M
  UNSURE (1)..(1): The 'Xaa' at location 1 stands for Lys or Arg
  UNSURE (8)..(8): The 'Xaa' at location 8 stands for Asn, Gly, Phe, Tyr, Ala, Asp, Leu, Met or Gln
  UNSURE (9)..(9): The 'Xaa' at location 9 stands for Ser or Thr
  UNSURE (10)..(10): The 'Xaa' at location 10 stands for Glu or Met
XIDPANGXXX

SEQ ID NO: 179 - protein, 9 aa, Artificial Sequence
  DOMAIN (1)..(9): Consensus humanized 29.39 VH CDR3 GNLHYX1LMD wherein X1=Y, A or G
  UNSURE (6)..(6): The 'Xaa' at location 6 stands for Tyr, Ala or Gly
GNLHYXLMD

SEQ ID NO: 180 - protein, 11 aa, Artificial Sequence
  DOMAIN (1)..(11): Consensus humanized 29.39 VL CDR1 KASQX1X2X3TYX4S wherein X1=A, P, or T; X2=I, T, or P; X3=N or A; X4=L, G or H
  UNSURE (5)..(5): The 'Xaa' at location 5 stands for Ala, Pro or Thr
  UNSURE (6)..(6): The 'Xaa' at location 6 stands for Ile, Thr or Pro
  UNSURE (7)..(7): The 'Xaa' at location 7 stands for Asn or Ala
  UNSURE (10)..(10): The 'Xaa' at location 10 stands for Leu,Gly or His
KASQXXXTYXS

SEQ ID NO: 181 - protein, 7 aa, Artificial Sequence
  DOMAIN (1)..(7): Consensus humanized 29.39 VL CDR2 RX1NRX2X3X4 wherein X1=A, Y, V, or D; X2=M, K, V, or A; X3=V, P, Y or G; X4=D or G
  UNSURE (2)..(2): The 'Xaa' at location 2 stands for Ala, Tyr, Val or Asp
  UNSURE (5)..(5): The 'Xaa' at location 5 stands for Met, Lys, Val or Ala
  UNSURE (6)..(6): The 'Xaa' at location 6 stands for Val, Pro, Tyr or Gly
  UNSURE (7)..(7): The 'Xaa' at location 7 stands for Asp or Gly
RXNRXXX

SEQ ID NO: 182 - protein, 9 aa, Artificial Sequence
  DOMAIN (1)..(9): Consensus humanized 29.39 VL CDR3 LQX1X2DFPYX3 wherein X1=Y, S, or F; X2=D, V, L, R, E or Q; X3=T or K
  UNSURE (3)..(3): The 'Xaa' at location 3 stands for Tyr, Ser or Phe
  UNSURE (4)..(4): The 'Xaa' at location 4 stands for Asp, Val, Leu, Arg, Glu or Gln
  UNSURE (9)..(9): The 'Xaa' at location 9 stands for Thr or Lys
LQXXDFPYX

SEQ ID NO: 183 - protein, 15 aa, Artificial Sequence
  DOMAIN (1)..(15): Exemplary linker183
GGGGSGGGGSGGGGS

SEQ ID NO: 184 - protein, 5 aa, Artificial Sequence
  DOMAIN (1)..(5): Exemplary linker184
GGGSG

SEQ ID NO: 185 - protein, 10 aa, Artificial Sequence
  DOMAIN (1)..(10): Exemplary linker185
GGGSGGGGSG

SEQ ID NO: 186 - protein, 12 aa, Artificial Sequence
  DOMAIN (1)..(12): Exemplary linker186
GSGGSGGSGGSG

SEQ ID NO: 187 - protein, 8 aa, Artificial Sequence
  DOMAIN (1)..(8): Exemplary linker187
GGSGGGSG

SEQ ID NO: 188 - protein, 12 aa, Artificial Sequence
  DOMAIN (1)..(12): Exemplary linker188
GGSGGGSGGGSG

SEQ ID NO: 189 - protein, 6 aa, Artificial Sequence
  DOMAIN (1)..(6): Exemplary linker189
GSGGSG

SEQ ID NO: 190 - protein, 9 aa, Artificial Sequence
  DOMAIN (1)..(9): Exemplary linker190
GSGGSGGSG

SEQ ID NO: 191 - protein, 7 aa, Artificial Sequence
  DOMAIN (1)..(7): Exemplary linker191
GSGSGSG

SEQ ID NO: 192 - protein, 18 aa, Artificial Sequence
  DOMAIN (1)..(18): Exemplary linker192
GGGGSGGGGSGGGGSGGG

SEQ ID NO: 193 - protein, 30 aa, Artificial Sequence
  DOMAIN (1)..(30): Exemplary linker193
GGGGSGGGGSGGGGSGGGGSGGGGSGGGGS

SEQ ID NO: 194 - protein, 5 aa, Artificial Sequence
  DOMAIN (1)..(5): Exemplary linker194
PAPAP

SEQ ID NO: 195 - protein, 15 aa, Artificial Sequence
  DOMAIN (1)..(15): Exemplary linker195
PAPAPPAPAPPAPAP

SEQ ID NO: 196 - protein, 7 aa, Artificial Sequence
  DOMAIN (1)..(7): Exemplary linker196
IKRTVAA

SEQ ID NO: 197 - protein, 7 aa, Artificial Sequence
  DOMAIN (1)..(7): Exemplary linker197
VSSASTK

SEQ ID NO: 198 - protein, 7 aa, Artificial Sequence
  DOMAIN (1)..(7): Exemplary linker198
AEAAAKA

SEQ ID NO: 199 - protein, 12 aa, Artificial Sequence
  DOMAIN (1)..(12): Exemplary linker199
AEAAAKEAAAKA

SEQ ID NO: 200 - protein, 10 aa, Artificial Sequence
  DOMAIN (1)..(10): Exemplary linker200
GRPGSGRPGS

SEQ ID NO: 201 - protein, 20 aa, Artificial Sequence
  DOMAIN (1)..(20): Exemplary linker201
GRPGSGRPGSGRPGSGRPGS

SEQ ID NO: 202 - protein, 10 aa, Artificial Sequence
  DOMAIN (1)..(10): Exemplary linker202
GRGGSGRGGS

SEQ ID NO: 203 - protein, 20 aa, Artificial Sequence
  DOMAIN (1)..(20): Exemplary linker203
GRGGSGRGGSGRGGSGRGGS

SEQ ID NO: 204 - protein, 10 aa, Artificial Sequence
  DOMAIN (1)..(10): Exemplary linker204
GKPGSGKPGS

SEQ ID NO: 205 - protein, 20 aa, Artificial Sequence
  DOMAIN (1)..(20): Exemplary linker205
GKPGSGKPGSGKPGSGKPGS

SEQ ID NO: 206 - protein, 10 aa, Artificial Sequence
  DOMAIN (1)..(10): Exemplary linker206
GEPGSGEPGS

SEQ ID NO: 207 - protein, 20 aa, Artificial Sequence
  DOMAIN (1)..(20): Exemplary linker
GEGGSGEGGSGEGGSGEGGS

SEQ ID NO: 208 - protein, 10 aa, Artificial Sequence
  DOMAIN (1)..(10): Exemplary linker208
GDPGSGDPGS

SEQ ID NO: 209 - protein, 20 aa, Artificial Sequence
  DOMAIN (1)..(20): Exemplary linker209
GDPGSGDPGSGDPGSGDPGS

SEQ ID NO: 210 - protein, 20 aa, Artificial Sequence
  DOMAIN (1)..(20): Exemplary linker210
GGGGSGGGGSGGGGSGGGGS

SEQ ID NO: 211 - protein, 5 aa, Artificial Sequence
  DOMAIN (1)..(5): Clone 2-9-1 VH CDR1
DTYIH

SEQ ID NO: 212 - protein, 17 aa, Artificial Sequence
  DOMAIN (1)..(17): Clone 2-9-1 VH CDR2
RIDPASGNSEYAQKFQG

SEQ ID NO: 213 - protein, 10 aa, Artificial Sequence
  DOMAIN (1)..(10): Clone 2-9-1 VH CDR3
GNLHYALMDY

SEQ ID NO: 214 - protein, 11 aa, Artificial Sequence
  DOMAIN (1)..(11): Clone 2-9-1 VL CDR1
KASQPINTYLS

SEQ ID NO: 215 - protein, 7 aa, Artificial Sequence
  DOMAIN (1)..(7): Clone 2-9-1 VL CDR2
RVNRKVD

SEQ ID NO: 216 - protein, 9 aa, Artificial Sequence
  DOMAIN (1)..(9): Clone 2-9-1 VL CDR3
LQYLDFPYT

SEQ ID NO: 217 - protein, 119 aa, Artificial Sequence
  DOMAIN (1)..(119): Clone 2-9-1 VH
QVQLVQSGAEVKKPGASVKASCKASGFNIQDTYIHWVRQAPGQGLEWMGRIDPASGNSEYAQKFQGRVTMTRDTSTSTVYMELSSLRSEDTAVYYCTTGNLHYALMDYWGQGTSVTVSS

SEQ ID NO: 218 - protein, 110 aa, Artificial Sequence; identical to SEQ ID NO: 128
  DOMAIN (1)..(110): Clone 2-9-1 VL

SEQ ID NO: 219 - protein, 449 aa, Artificial Sequence
  CHAIN (1)..(449): Clone 2-9-1 HC
QVQLVQSGAEVKKPGASVKASCKASGFNIQDTYIHWVRQAPGQGLEWMGRIDPASGNSEYAQKFQGRVTMTRDTSTSTVYMELSSLRSEDTAVYYCTTGNLHYALMDYWGQGTSVTVSSASTKGPSVFPLAPSSKSTSGGTAALGCLVKDYFPEPVTVSWNSGALTSGVHTFPAVLQSSGLYSLSSVVTVPSSSLGTQTYICNVNHKPSNTKVDKKVEPKSCDKTHTCPPCPAPELLGGPSVFLFPPKPKDTLMISRTPEVTCVVVDVEHEDPEVKFNWYVDGVEVHNAKTKPREEQYNSTYRVVSVLTVLHQDWLNGKEYKCKVSNKAFPAPIEKTISKAKGQPREPQVYTLPPSREEMTKNQVSLTCLVKGFYPSDIAVEWESNGQPENNYKTTPPVLDSDGSFFLYSKLTVDKSRWQQGNVFSCSVMHEALHNHYTQKSLSLSPGK

SEQ ID NO: 220 - protein, 214 aa, Artificial Sequence; identical to SEQ ID NO: 130
  DOMAIN (1)..(214): Clone 2-9-1 LC

SEQ ID NO: 221 - protein, 5 aa, Artificial Sequence
  DOMAIN (1)..(5): Clone 2-9-2 VH CDR1
DTYIH

SEQ ID NO: 222 - protein, 17 aa, Artificial Sequence
  DOMAIN (1)..(17): Clone 2-9-2 VH CDR2
RIDPASGNSEYAQKFQG

SEQ ID NO: 223 - protein, 10 aa, Artificial Sequence
  DOMAIN (1)..(10): Clone 2-9-2 VH CDR3
GNLHYALMDY

SEQ ID NO: 224 - protein, 11 aa, Artificial Sequence
  DOMAIN (1)..(11): Clone 2-9-2 VL CDR1
KASQPINTYLS

SEQ ID NO: 225 - protein, 7 aa, Artificial Sequence
  DOMAIN (1)..(7): Clone 2-9-2 VL CDR2
RVNRKVD

SEQ ID NO: 226 - protein, 9 aa, Artificial Sequence
  DOMAIN (1)..(9): Clone 2-9-2 VL CDR3
LQYLDFPYT

SEQ ID NO: 227 - protein, 119 aa, Artificial Sequence
  DOMAIN (1)..(119): Clone 2-9-2 VH
QVQLVQSGAEVKKPGASVKVSCKASGFNIQDTYIHWVRQAPGQGLEWMGRIDPASGNSEYAQKFQGRVTMTRDTSTSTVYMELSSLRSEDTAVYYCTTGNLHYALMDYWGQGTSVTVSS

SEQ ID NO: 228 - protein, 110 aa, Artificial Sequence; identical to SEQ ID NO: 128
  DOMAIN (1)..(228): Clone 2-9-2 VL

SEQ ID NO: 229 - protein, 446 aa, Artificial Sequence
  CHAIN (1)..(446): Clone 2-9-2 HC
QVQLVQSGAEVKKPGASVKVSCKASGFNIQDTYIHWVRQAPGQGLEWMGRIDPASGNSEYAQKFQGRVTMTRDTSTSTVYMELSSLRSEDTAVYYCTTGNLHYALMDYWGQGTSVTVSSASTKGPSVFPLAPCSRSTSESTAALGCLVKDYFPEPVTVSWNSGALTSGVHTFPAVLQSSGLYSLSSVVTVPSSSLGTKTYTCNVDHKPSNTKVDKRVESKYGPPCPPCPAPEFLGGPSVFLFPPKPKDTLMISRTPEVTCVVVDVSQEDPEVQFNWYVDGVEVHNAKTKPREEQFNSTYRVVSVLTVLHQDWLNGKEYKCKVSNKGLPSSIEKTISKAKGQPREPQVYTLPPSQEEMTKNQVSLTCLVKGFYPSDIAVEWESNGQPENNYKTTPPVLDSDGSFFLYSRLTVDKSRWQEGNVFSCSVMHEALHNHYTQKSLSLSLGK

SEQ ID NO: 230 - protein, 214 aa, Artificial Sequence; identical to SEQ ID NO: 130
  CHAIN (1)..(214): Clone 2-9-2 LC